European Patent Application EP 4 707 296 A1, published March 11, 2026. Title: INTERLEUKIN-2 VARIANTS WITH MODIFIED BIOLOGICAL ACTIVITY. Applicant: EGLE THERAPEUTICS. Application EP. The sequence listing filed with the application follows.

SEQUENCE LISTING (12 sequences)

SEQ ID NO: 1 - protein, 133 aa, Homo sapiens [sequence omitted]

SEQ ID NO: 2 - protein, 132 aa, synthetic construct
APTSSTKKTQLQLERLLLDLQMILNGINNYKNPKLTRMLTFKFYMPKKATELKHLQCLEEELKPLEEVLNLAQSKNFHLRPRDLISNINVIVLELKGSETTFMCEYADETATIVEFLNRWITFCQSIISTLT

SEQ ID NO: 3 - protein, 132 aa, synthetic construct
APTSSTKKTQLQLERLLRDLQMILNGINNYKNPKLTRMLTFKFYMPKKATELKHLQCLEEELKPLEEVLNLAQSKNFHLRPRDLISNINVIVLELKGSETTFMCEYADETATIVEFLNRWITFCQSIISTLT

SEQ ID NO: 4 - protein, 132 aa, synthetic construct
APTSSTKKTQLQLERLLLDLQMILNGINNYKNPKLTRMLTFKFYMPKKATELKHLQCLEEELKPLEEVLNLAQSKNFHLRPRDLISNINKIVLELKGSETTFMCEYADETATIVEFLNRWITFCQSIISTLT

SEQ ID NO: 5 - protein, 132 aa, synthetic construct
APTSSTKKTQLQLEHLLRDLQMILNGINNYKNPKLTRMLTFKFYMPKKATELKHLQCLEEELKPLEEVLNLAQSKNFHLRPRDLISNINKIVLELKGSETTFMCEYADETATIVEFLNRWITFCQSIISTLT

SEQ ID NO: 6 - protein, 132 aa, synthetic construct
APTSSTKKTQLQLERLLRDLQMILNGINNYKNPKLTRMLTFKFYMPKKATELKHLQCLEEELKPLEEVLNLAQSKNFHLRPRDLISNINKIVLELKGSETTFMCEYADETATIVEFLNRWITFCQSIISTLT

SEQ ID NO: 7 - protein, 15 aa, synthetic construct
GGGGSGGGGSGGGGS

SEQ ID NO: 8 - DNA, 396 bp, synthetic construct
  source 1..396: mol_type = other DNA
gcgcccaccagtagcaccaaaaagacccagctgcaattagagcggctgttgctggatctgcaaatgatactgaacggcattaacaactataaaaatcccaagctgacgaggatgctgacattcaagttctacatgcccaagaaggctactgaactgaaacacctgcaatgcttggaggaagagctgaagccactggaggaagtgctcaatttagcacagagcaagaactttcaccttcggccgcgggatctgatctctaatattaatgtcatagtcctggagttaaaggggagtgaaactacatttatgtgcgaatatgccgacgaaacagcaactatagtcgagtttctgaacaggtggatcacattttgccagtctatcatctctactctgact

SEQ ID NO: 9 - DNA, 396 bp, synthetic construct
  source 1..396: mol_type = other DNA
gccccaacttcttcaaccaagaagactcagctccagttggagcgactgctacgtgacctccagatgattctgaatgggatcaataactataaaaatccaaagctgactaggatgcttacatttaagttttatatgcctaagaaggcgaccgagctcaagcatttacagtgtctggaagaggagctgaagcctttggaggaagtcttgaatctggctcaatccaagaattttcacctgagacccagggatttgatttcaaacatcaacgtgattgtgttagagctgaagggttctgagaccacatttatgtgtgagtacgctgacgaaaccgctaccattgtggaatttctgaacagatggattacattctgtcagtcaatcatcagcaccctgacc

SEQ ID NO: 10 - DNA, 396 bp, synthetic construct
  source 1..396: mol_type = other DNA
gcacccaccagttcgaccaaaaagacgcagctgcaattagagcggctgttactggatctgcaaatgatactgaacggcattaacaactataaaaatcccaagctgacaaggatgctgacattcaagttctacatgcccaagaaggccactgaactgaaacacctgcaatgcttggaggaagagctgaagccactagaggaggtgctcaatttagcacagtcgaagaactttcaccttcggccgcgggacctgatctctaatattaataaaatagtcctggagctgaaggggagcgaaactacatttatgtgcgagtatgccgatgaaacagcaactatagtcgagtttctgaacaggtggatcacattttgccagtctatcatctctactctgact

SEQ ID NO: 11 - DNA, 396 bp, synthetic construct
  source 1..396: mol_type = other DNA
gcgccaacctcaagtacaaaaaagacacagctgcaactggagcatctgcttcgagacctgcaaatgatcctgaatggcattaacaactataaaaacccaaaattaacaaggatgctgactttcaagttttacatgcctaagaaggccacagaactgaaacatctgcaatgtctggaggaggagttgaagccactggaggaggtcctaaacctggcacagtctaagaattttcatctgaggccgcgggatctaatctccaatataaataaaatagtccttgagctgaaaggaagcgagacaacttttatgtgcgaatatgctgacgagaccgctaccatagtcgagtttctgaatagatggattactttctgccaaagtataatttcaaccctgacc

SEQ ID NO: 12 - DNA, 396 bp, synthetic construct
  source 1..396: mol_type = other DNA
gcgcctaccagcagtaccaagaaaacccagctgcaactggagaggctgctgcgggacctgcaaatgattctgaacggtatcaacaactacaaaaatcctaaacttacacgtatgctgacctttaaattttacatgcctaaaaaggccaccgagctcaagcatctgcaatgcttggaggaagagctcaagccgctggaagaggtgctgaatttggcccaatccaagaacttccacctgcggcctcgcgacctgatcagcaacattaataaaatcgtgttggaactgaagggcagtgagactacgtttatgtgtgagtacgctgacgagaccgcgaccattgtcgagtttctgaatagatggatcacattttgtcagtccatcatttcgacgctgact